European Patent Application EP 4 660 201 A1, published December 10, 2025. Title: 抗原结合蛋白及其用途. Applicant: 北京可瑞生物科技有限公司. Application CN. The sequence listing filed with the application follows.

SEQUENCE LISTING (110 sequences)

SEQ ID NO: 1-18 - skipped (18 entries)

SEQ ID NO: 19 - protein, 19 aa, Artificial Sequence
MASAPISMLAMLFTLSGLR

SEQ ID NO: 20 - protein, 19 aa, Artificial Sequence
MDSWTFCCVSLCILVAKHT

SEQ ID NO: 21 - protein, 21 aa, Artificial Sequence
MISLRVLLVILWLQLSWVWSQ

SEQ ID NO: 22 - protein, 15 aa, Artificial Sequence
AVRDIEGAGNNRKLI

SEQ ID NO: 23 - protein, 13 aa, Artificial Sequence
VVPGGTGGGNKLT

SEQ ID NO: 24 - protein, 13 aa, Artificial Sequence
AENSDGTSYGKLT

SEQ ID NO: 25 - protein, 12 aa, Artificial Sequence
AVNLGAAGNKLT

SEQ ID NO: 26 - protein, 8 aa, Artificial Sequence
VVTNARLM

SEQ ID NO: 27 - protein, 6 aa, human
VSGNPY

SEQ ID NO: 28 - protein, 6 aa, human
NSASQS

SEQ ID NO: 29 - protein, 6 aa, human
NSASDY

SEQ ID NO: 30 - protein, 6 aa, human
DRGSQS

SEQ ID NO: 31 - protein, 6 aa, human
NSASQS

SEQ ID NO: 32 - protein, 8 aa, human
YITGDNLV

SEQ ID NO: 33 - protein, 6 aa, human
VYSSGN

SEQ ID NO: 34 - protein, 7 aa, human
IRSNMDK

SEQ ID NO: 35 - protein, 6 aa, human
IYSNGD

SEQ ID NO: 36 - protein, 6 aa, human
VYSSGN

SEQ ID NO: 37 - protein, 11 aa, human
ASSEGFYTEAF

SEQ ID NO: 38 - protein, 12 aa, human
ASSHWGAQETQY

SEQ ID NO: 39 - protein, 13 aa, human
ASSLVGSPDYEQY

SEQ ID NO: 40 - protein, 13 aa, human
ASSFSDSYNSPLH

SEQ ID NO: 41 - protein, 14 aa, human
ASTSIVSSGRGEQF

SEQ ID NO: 42 - protein, 5 aa, human
SGHNS

SEQ ID NO: 43 - protein, 5 aa, human
LGHDT

SEQ ID NO: 44 - protein, 5 aa, human
SGHAT

SEQ ID NO: 45 - protein, 5 aa, human
SGHAT

SEQ ID NO: 46 - protein, 5 aa, human
MNHEY

SEQ ID NO: 47 - protein, 6 aa, human
FNNNVP

SEQ ID NO: 48 - protein, 6 aa, human
YNNKEL

SEQ ID NO: 49 - protein, 6 aa, human
FQNNGV

SEQ ID NO: 50 - protein, 6 aa, human
FQNNGV

SEQ ID NO: 51 - protein, 6 aa, human
SMNVEV

SEQ ID NO: 52 - protein, 117 aa, human
AQSVAQPEDQVNVAEGNPLTVKCTYSVSGNPYLFWYVQYPNRGLQFLLKYITGDNLVKGSYGFEAEFNKSQTSFHLKKPSALVSDSALYFCAVRDIEGAGNNRKLIWGLGTSLAVNP

SEQ ID NO: 53 - protein, 112 aa, human
RKEVEQDPGPFNVPEGATVAFNCTYSNSASQSFFWYRQDCRKEPKLLMSVYSSGNEDGRFTAQLNRASQYISLLIRDSKLSDSATYLCVVPGGTGGGNKLTFGTGTQLKVEL

SEQ ID NO: 54 - protein, 114 aa, human
GESVGLHLPTLGVQEGDNSIINCAYSNSASDYFIWYKQESGKGPQFIIDIRSNMDKRQGQRVTVLLNKTVKHLSLQIAATQPGDSAVYFCAENSDGTSYGKLTFGQGTILTVHP

SEQ ID NO: 55 - protein, 112 aa, human
QKEVEQNSGPLSVPEGAIASLNCTYSDRGSQSFFWYRQYSGKSPELIMSIYSNGDKEDGRFTAQLNKASQYVSLLIRDSQPSDSATYLCAVNLGAAGNKLTFGGGTRVLVKP

SEQ ID NO: 56 - protein, 107 aa, human
RKEVEQDPGPFNVPEGATVAFNCTYSNSASQSFFWYRQDCRKEPKLLMSVYSSGNEDGRFTAQLNRASQYISLLIRDSKLSDSATYLCVVTNARLMFGDGTQLVVKP

SEQ ID NO: 57 - protein, 113 aa, human
DAGVIQSPRHEVTEMGQEVTLRCKPISGHNSLFWYRQTMMRGLELLIYFNNNVPIDDSGMPEDRFSAKMPNASFSTLKIQPSEPRDSAVYFCASSEGFYTEAFFGQGTRLTVV

SEQ ID NO: 58 - protein, 113 aa, human
DTAVSQTPKYLVTQMGNDKSIKCEQNLGHDTMDWYKQDSKKFLKIMFSYNNKELIINETVPNRFSPKSPDKAHLNLHINSLELGDSAVYFCASSHWGAQETQYFGPGTRLLVL

SEQ ID NO: 59 - protein, 115 aa, human
EAGVAQSPRYKIIEKRQSVAFWCNPISGHATLYWYQQILGQGPKLLIQFQNNGVVDDSQLPKDRFSAERLKGVDSTLKIQPAKLEDSAVYLCASSLVGSPDYEQYFGPGTRLTVT

SEQ ID NO: 60 - protein, 115 aa, human
EAGVAQSPRYKIIEKRQSVAFWCNPISGHATLYWYQQILGQGPKLLIQFQNNGVVDDSQLPKDRFSAERLKGVDSTLKIQPAKLEDSAVYLCASSFSDSYNSPLHFGNGTRLTVT

SEQ ID NO: 61 - protein, 115 aa, human
EAQVTQNPRYLITVTGKKLTVTCSQNMNHEYMSWYRQDPGLGLRQIYYSMNVEVTDKGDVPEGYKVSRKEKRNFPLILESPSPNQTSLYFCASTSIVSSGRGEQFFGPGTRLTVL

SEQ ID NO: 62 - protein, 141 aa, human
NIQNPDPAVYQLRDSKSSDKSVCLFTDFDSQTNVSQSKDSDVYITDKTVLDMRSMDFKSNSAVAWSNKSDFACANAFNNSIIPEDTFFPSPESSCDVKLVEKSFETDTNLNFQNLSVIGFRILLLKVAGFNLLMTLRLWSS

SEQ ID NO: 63 - protein, 141 aa, human
NIQNPDPAVYQLRDSKSSDKSVCLFTDFDSQTNVSQSKDSDVYITDKCVLDMRSMDFKSNSAVAWSNKSDFACANAFNNSIIPEDTFFPSPESSCDVKLVEKSFETDTNLNFQNLSVIGFRILLLKVAGFNLLMTLRLWSS

SEQ ID NO: 64 - protein, 141 aa, human
NIQNPDPAVYQLRDSKSSDKSVCLFTDFDSQTNVSQSKDSDVYITDKCVLDMRSMDFKSNSAVAWSNKSDFACANAFNNSIIPEDTFFPSPESSCDVKLVEKSFETDTNLNFQNLLVIVLRILLLKVAGFNLLMTLRLWSS

SEQ ID NO: 65 - protein, 137 aa, mouse
NIQNPEPAVYQLKDPRSQDSTLCLFTDFDSQINVPKTMESGTFITDKTVLDMKAMDSKSNGAIAWSNQTSFTCQDIFKETNATYPSSDVPCDATLTEKSFETDMNLNFQNLSVMGLRILLLKVAGFNLLMTLRLWSS

SEQ ID NO: 66 - protein, 137 aa, mouse
NIQNPEPAVYQLKDPRSQDSTLCLFTDFDSQINVPKTMESGTFITDKCVLDMKAMDSKSNGAIAWSNQTSFTCQDIFKETNATYPSSDVPCDATLTEKSFETDMNLNFQNLLVIVLRILLLKVAGFNLLMTLRLWSS

SEQ ID NO: 67 - protein, 177 aa, human
EDLNKVFPPEVAVFEPSEAEISHTQKATLVCLATGFFPDHVELSWWVNGKEVHSGVSTDPQPLKEQPALNDSRYCLSSRLRVSATFWQNPRNHFRCQVQFYGLSENDEWTQDRAKPVTQIVSAEAWGRADCGFTSVSYQQGVLSATILYEILLGKATLYAVLVSALVLMAMVKRKDF

SEQ ID NO: 68 - protein, 177 aa, human
EDLNKVFPPEVAVFEPSEAEISHTQKATLVCLATGFFPDHVELSWWVNGKEVHSGVCTDPQPLKEQPALNDSRYCLSSRLRVSATFWQNPRNHFRCQVQFYGLSENDEWTQDRAKPVTQIVSAEAWGRADCGFTSVSYQQGVLSATILYEILLGKATLYAVLVSALVLMAMVKRKDF

SEQ ID NO: 69 - protein, 179 aa, human
EDLKNVFPPKVAVFEPSEAEISHTQKATLVCLATGFYPDHVELSWWVNGKEVHSGVSTDPQPLKEQPALNDSRYCLSSRLRVSATFWQNPRNHFRCQVQFYGLSENDEWTQDRAKPVTQIVSAEAWGRADCGFTSESYQQGVLSATILYEILLGKATLYAVLVSALVLMAMVKRKDSRG

SEQ ID NO: 70 - protein, 179 aa, human
EDLKNVFPPKVAVFEPSEAEISHTQKATLVCLATGFYPDHVELSWWVNGKEVHSGVCTDPQPLKEQPALNDSRYCLSSRLRVSATFWQNPRNHFRCQVQFYGLSENDEWTQDRAKPVTQIVSAEAWGRADCGFTSESYQQGVLSATILYEILLGKATLYAVLVSALVLMAMVKRKDSRG

SEQ ID NO: 71 - protein, 173 aa, mouse
EDLRNVTPPKVSLFEPSKAEIANKQKATLVCLARGFFPDHVELSWWVNGKEVHSGVSTDPQAYKESNYSYCLSSRLRVSATFWHNPRNHFRCQVQFHGLSEEDKWPEGSPKPVTQNISAEAWGRADCGITSASYQQGVLSATILYEILLGKATLYAVLVSTLVVMAMVKRKNS

SEQ ID NO: 72 - protein, 173 aa, mouse
EDLRNVTPPKVSLFEPSKAEIANKQKATLVCLARGFFPDHVELSWWVNGKEVHSGVCTDPQAYKESNYSYCLSSRLRVSATFWHNPRNHFRCQVQFHGLSEEDKWPEGSPKPVTQNISAEAWGRADCGITSASYQQGVLSATILYEILLGKATLYAVLVSTLVVMAMVKRKNS

SEQ ID NO: 73 - protein, 171 aa, mouse
EDLRNVTPPKVSLFEPSKAEIANKQKATLVCLARGFFPDHVELSWWVNGKEVHSGVSTDPQAYKESNYSYCLSSRLRVSATFWHNPRNHFRCQVQFHGLSEEDKWPEGSPKPVTQNISAEAWGRADCGITSASYQQGVLSATILYEILLGKATLYAVLVSTLVVMAMVRNR

SEQ ID NO: 74 - protein, 171 aa, mouse
EDLRNVTPPKVSLFEPSKAEIANKQKATLVCLARGFFPDHVELSWWVNGKEVHSGVCTDPQAYKESNYSYCLSSRLRVSATFWHNPRNHFRCQVQFHGLSEEDKWPEGSPKPVTQNISAEAWGRADCGITSASYQQGVLSATILYEILLGKATLYAVLVSTLVVMAMVRNR

SEQ ID NO: 75 - protein, 173 aa, mouse
EDLRNVTPPKVSLFEPSKAEIANKQKATLVCLARGFFPDHVELSWWVNGKEVHSGVSTDPQAYKESNYSYCLSSRLRVSATFWHNPRNHFRCQVQFHGLSEEDKWPEGSPKPVTQNISAEAWGRADCGITSASYHQGVLSATILYEILLGKATLYAVLVSGLVLMAMVKKKNS

SEQ ID NO: 76 - protein, 173 aa, mouse
EDLRNVTPPKVSLFEPSKAEIANKQKATLVCLARGFFPDHVELSWWVNGKEVHSGVCTDPQAYKESNYSYCLSSRLRVSATFWHNPRNHFRCQVQFHGLSEEDKWPEGSPKPVTQNISAEAWGRADCGITSASYHQGVLSATILYEILLGKATLYAVLVSGLVLMAMVKKKNS

SEQ ID NO: 77 - protein, 273 aa, Artificial Sequence
MASAPISMLAMLFTLSGLRAQSVAQPEDQVNVAEGNPLTVKCTYSVSGNPYLFWYVQYPNRGLQFLLKYITGDNLVKGSYGFEAEFNKSQTSFHLKKPSALVSDSALYFCAVRDIEGAGNNRKLIWGLGTSLAVNPNIQNPEPAVYQLKDPRSQDSTLCLFTDFDSQINVPKTMESGTFITDKCVLDMKAMDSKSNGAIAWSNQTSFTCQDIFKETNATYPSSDVPCDATLTEKSFETDMNLNFQNLLVIVLRILLLKVAGFNLLMTLRLWSS

SEQ ID NO: 78 - protein, 270 aa, Artificial Sequence
MISLRVLLVILWLQLSWVWSQRKEVEQDPGPFNVPEGATVAFNCTYSNSASQSFFWYRQDCRKEPKLLMSVYSSGNEDGRFTAQLNRASQYISLLIRDSKLSDSATYLCVVPGGTGGGNKLTFGTGTQLKVELNIQNPEPAVYQLKDPRSQDSTLCLFTDFDSQINVPKTMESGTFITDKCVLDMKAMDSKSNGAIAWSNQTSFTCQDIFKETNATYPSSDVPCDATLTEKSFETDMNLNFQNLLVIVLRILLLKVAGFNLLMTLRLWSS

SEQ ID NO: 79 - protein, 271 aa, Artificial Sequence
MAGIRALFMYLWLQLDWVSRGESVGLHLPTLGVQEGDNSIINCAYSNSASDYFIWYKQESGKGPQFIIDIRSNMDKRQGQRVTVLLNKTVKHLSLQIAATQPGDSAVYFCAENSDGTSYGKLTFGQGTILTVHPNIQNPEPAVYQLKDPRSQDSTLCLFTDFDSQINVPKTMESGTFITDKCVLDMKAMDSKSNGAIAWSNQTSFTCQDIFKETNATYPSSDVPCDATLTEKSFETDMNLNFQNLLVIVLRILLLKVAGFNLLMTLRLWSS

SEQ ID NO: 80 - protein, 271 aa, Artificial Sequence
MMKSLRVLLVILWLQLSWVWSQQKEVEQNSGPLSVPEGAIASLNCTYSDRGSQSFFWYRQYSGKSPELIMSIYSNGDKEDGRFTAQLNKASQYVSLLIRDSQPSDSATYLCAVNLGAAGNKLTFGGGTRVLVKPNIQNPEPAVYQLKDPRSQDSTLCLFTDFDSQINVPKTMESGTFITDKCVLDMKAMDSKSNGAIAWSNQTSFTCQDIFKETNATYPSSDVPCDATLTEKSFETDMNLNFQNLLVIVLRILLLKVAGFNLLMTLRLWSS

SEQ ID NO: 81 - protein, 265 aa, Artificial Sequence
MISLRVLLVILWLQLSWVWSQRKEVEQDPGPFNVPEGATVAFNCTYSNSASQSFFWYRQDCRKEPKLLMSVYSSGNEDGRFTAQLNRASQYISLLIRDSKLSDSATYLCVVTNARLMFGDGTQLVVKPNIQNPEPAVYQLKDPRSQDSTLCLFTDFDSQINVPKTMESGTFITDKCVLDMKAMDSKSNGAIAWSNQTSFTCQDIFKETNATYPSSDVPCDATLTEKSFETDMNLNFQNLLVIVLRILLLKVAGFNLLMTLRLWSS

SEQ ID NO: 82 - protein, 305 aa, Artificial Sequence
MDSWTFCCVSLCILVAKHTDAGVIQSPRHEVTEMGQEVTLRCKPISGHNSLFWYRQTMMRGLELLIYFNNNVPIDDSGMPEDRFSAKMPNASFSTLKIQPSEPRDSAVYFCASSEGFYTEAFFGQGTRLTVVEDLRNVTPPKVSLFEPSKAEIANKQKATLVCLARGFFPDHVELSWWVNGKEVHSGVCTDPQAYKESNYSYCLSSRLRVSATFWHNPRNHFRCQVQFHGLSEEDKWPEGSPKPVTQNISAEAWGRADCGITSASYQQGVLSATILYEILLGKATLYAVLVSTLVVMAMVKRKNS

SEQ ID NO: 83 - protein, 305 aa, Artificial Sequence
MGCRLLCCVVFCLLQAGPLDTAVSQTPKYLVTQMGNDKSIKCEQNLGHDTMDWYKQDSKKFLKIMFSYNNKELIINETVPNRFSPKSPDKAHLNLHINSLELGDSAVYFCASSHWGAQETQYFGPGTRLLVLEDLRNVTPPKVSLFEPSKAEIANKQKATLVCLARGFFPDHVELSWWVNGKEVHSGVCTDPQAYKESNYSYCLSSRLRVSATFWHNPRNHFRCQVQFHGLSEEDKWPEGSPKPVTQNISAEAWGRADCGITSASYQQGVLSATILYEILLGKATLYAVLVSTLVVMAMVKRKNS

SEQ ID NO: 84 - protein, 307 aa, Artificial Sequence
MSTRLLCWAALCLLGAELTEAGVAQSPRYKIIEKRQSVAFWCNPISGHATLYWYQQILGQGPKLLIQFQNNGVVDDSQLPKDRFSAERLKGVDSTLKIQPAKLEDSAVYLCASSLVGSPDYEQYFGPGTRLTVTEDLRNVTPPKVSLFEPSKAEIANKQKATLVCLARGFFPDHVELSWWVNGKEVHSGVCTDPQAYKESNYSYCLSSRLRVSATFWHNPRNHFRCQVQFHGLSEEDKWPEGSPKPVTQNISAEAWGRADCGITSASYQQGVLSATILYEILLGKATLYAVLVSTLVVMAMVKRKNS

SEQ ID NO: 85 - protein, 307 aa, Artificial Sequence
MSTRLLCWAALCLLGAELTEAGVAQSPRYKIIEKRQSVAFWCNPISGHATLYWYQQILGQGPKLLIQFQNNGVVDDSQLPKDRFSAERLKGVDSTLKIQPAKLEDSAVYLCASSFSDSYNSPLHFGNGTRLTVTEDLRNVTPPKVSLFEPSKAEIANKQKATLVCLARGFFPDHVELSWWVNGKEVHSGVCTDPQAYKESNYSYCLSSRLRVSATFWHNPRNHFRCQVQFHGLSEEDKWPEGSPKPVTQNISAEAWGRADCGITSASYQQGVLSATILYEILLGKATLYAVLVSTLVVMAMVKRKNS

SEQ ID NO: 86 - protein, 307 aa, Artificial Sequence
MGPQLLGYVVLCLLGAGPLEAQVTQNPRYLITVTGKKLTVTCSQNMNHEYMSWYRQDPGLGLRQIYYSMNVEVTDKGDVPEGYKVSRKEKRNFPLILESPSPNQTSLYFCASTSIVSSGRGEQFFGPGTRLTVLEDLRNVTPPKVSLFEPSKAEIANKQKATLVCLARGFFPDHVELSWWVNGKEVHSGVCTDPQAYKESNYSYCLSSRLRVSATFWHNPRNHFRCQVQFHGLSEEDKWPEGSPKPVTQNISAEAWGRADCGITSASYQQGVLSATILYEILLGKATLYAVLVSTLVVMAMVKRKNS

SEQ ID NO: 87 - DNA, 351 bp, Artificial Sequence
  source 1..351: mol_type = other DNA
gctcagtcagtggctcagccggaagatcaggtcaacgttgctgaagggaatcctctgactgtgaaatgcacctattcagtctctggaaacccttatcttttttggtatgttcaataccccaaccgaggcctccagttccttctgaaatacatcacaggggataacctggttaaaggcagctatggctttgaagctgaatttaacaagagccaaacctccttccacctgaagaaaccatctgcccttgtgagcgactccgctttgtacttctgtgctgtgagagacatcgagggggctggcaacaaccgtaagctgatttggggattgggaacaagcctggcagtaaatccg

SEQ ID NO: 88 - DNA, 336 bp, Artificial Sequence
  source 1..336: mol_type = other DNA
cggaaggaggtggagcaggatcctggacccttcaatgttccagagggagccactgtcgctttcaactgtacttacagcaacagtgcttctcagtctttcttctggtacagacaggattgcaggaaagaacctaagttgctgatgtccgtatactccagtggtaatgaagatggaaggtttacagcacagctcaatagagccagccagtatatttccctgctcatcagagactccaagctcagtgattcagccacctacctctgtgtggtccctgggggcacgggaggaggaaacaaactcacctttgggacaggcactcagctaaaagtggaactc

SEQ ID NO: 89 - DNA, 342 bp, Artificial Sequence
  source 1..342: mol_type = other DNA
ggagagagtgtggggctgcatcttcctaccctgggtgtccaggagggtgacaactctattatcaactgtgcttattcaaacagcgcctcagactacttcatttggtacaagcaagaatctggaaaaggtcctcaattcattatagacattcgttcaaatatggacaaaaggcaaggccaaagagtcaccgttttattgaataagacagtgaaacatctctctctgcaaattgcagctactcaacctggagactcagctgtctacttttgtgcagagaattcggatggtactagctatggaaagctgacatttggacaagggaccatcttgactgtccatcca

SEQ ID NO: 90 - DNA, 336 bp, Artificial Sequence
  source 1..336: mol_type = other DNA
cagaaggaggtggagcagaattctggacccctcagtgttccagagggagccattgcctctctcaactgcacttacagtgaccgaggttcccagtccttcttctggtacagacaatattctgggaaaagccctgagttgataatgtccatatactccaatggtgacaaagaagatggaaggtttacagcacagctcaataaagccagccagtatgtttctctgctcatcagagactcccagcccagtgattcagccacctacctctgtgccgtgaacttgggggctgcaggcaacaagctaacttttggaggaggaaccagggtgctagttaaacca

SEQ ID NO: 91 - DNA, 321 bp, Artificial Sequence
  source 1..321: mol_type = other DNA
cggaaggaggtggagcaggatcctggacccttcaatgttccagagggagccactgtcgctttcaactgtacttacagcaacagtgcttctcagtctttcttctggtacagacaggattgcaggaaagaacctaagttgctgatgtccgtatactccagtggtaatgaagatggaaggtttacagcacagctcaatagagccagccagtatatttccctgctcatcagagactccaagctcagtgattcagccacctacctctgtgtggtgacaaatgccagactcatgtttggagatggaactcagctggtggtgaagccc

SEQ ID NO: 92 - DNA, 339 bp, Artificial Sequence
  source 1..339: mol_type = other DNA
gatgctggagttatccagtcaccccgccatgaggtgacagagatgggacaagaagtgactctgagatgtaaaccaatttcaggccacaactcccttttctggtacagacagaccatgatgcggggactggagttgctcatttactttaacaacaacgttccgatagatgattcagggatgcccgaggatcgattctcagctaagatgcctaatgcatcattctccactctgaagatccagccctcagaacccagggactcagctgtgtacttctgtgccagcagtgaggggttttacactgaagctttctttggacaaggcaccagactcacagttgta

SEQ ID NO: 93 - DNA, 339 bp, Artificial Sequence
  source 1..339: mol_type = other DNA
gacacagctgtttcccagactccaaaatacctggtcacacagatgggaaacgacaagtccattaaatgtgaacaaaatctgggccatgatactatggattggtataaacaggactctaagaaatttctgaagataatgtttagctacaataataaggagctcattataaatgaaacagttccaaatcgcttctcacctaaatctccagacaaagctcacttaaatcttcacatcaattccctggagcttggtgactctgctgtgtatttctgtgccagcagccattggggggcgcaggagacccagtacttcgggccaggcacgcggctcctggtgctc

SEQ ID NO: 94 - DNA, 345 bp, Artificial Sequence
  source 1..345: mol_type = other DNA
gaagctggagttgcccagtctcccagatataagattatagagaaaaggcagagtgtggctttttggtgcaatcctatatctggccatgctaccctttactggtaccagcagatcctgggacagggcccaaagcttctgattcagtttcagaataacggtgtagtggatgattcacagttgcctaaggatcgattttctgcagagaggctcaaaggagtagactccactctcaagatccagcctgcaaagcttgaggactcggccgtgtatctctgtgccagcagcttagttggcagtcctgattacgagcagtacttcgggccgggcaccaggctcacggtcaca

SEQ ID NO: 95 - DNA, 345 bp, Artificial Sequence
  source 1..345: mol_type = other DNA
gaagctggagttgcccagtctcccagatataagattatagagaaaaggcagagtgtggctttttggtgcaatcctatatctggccatgctaccctttactggtaccagcagatcctgggacagggcccaaagcttctgattcagtttcagaataacggtgtagtggatgattcacagttgcctaaggatcgattttctgcagagaggctcaaaggagtagactccactctcaagatccaacctgcaaagcttgaggactcggccgtgtatctctgtgccagcagcttctcggattcctataattcacccctccactttgggaacgggaccaggctcactgtgaca

SEQ ID NO: 96 - DNA, 345 bp, Artificial Sequence
  source 1..345: mol_type = other DNA
gaagcccaagtgacccagaacccaagatacctcatcacagtgactggaaagaagttaacagtgacttgttctcagaatatgaaccatgagtatatgtcctggtatcgacaagacccagggctgggcttaaggcagatctactattcaatgaatgttgaggtgactgataagggagatgttcctgaagggtacaaagtctctcgaaaagagaagaggaatttccccctgatcctggagtcgcccagccccaaccagacctctctgtacttctgtgccagcacctctattgtgagtagcgggaggggcgagcagttcttcgggccagggacacggctcaccgtgcta

SEQ ID NO: 97 - DNA, 411 bp, mouse
  source 1..411: mol_type = other DNA
aatattcagaaccccgaaccagccgtatatcagttgaaggacccaagatctcaggatagtacactctgcctgttcaccgactttgactcacaaatcaacgtcccgaagactatggaaagtggtacgttcatcacagataagtgcgttctggacatgaaggctatggactcaaagagcaacggggcaattgcttggtccaaccagacaagctttacctgtcaggacatttttaaggagactaatgctacttatccctccagcgacgttccgtgtgatgcgactcttaccgagaagtcttttgagaccgatatgaatctcaacttccagaatctgctggtgatcgttctgcggatcctgcttctgaaggttgcaggattcaatcttcttatgactctccggctctggtcttca

SEQ ID NO: 98 - DNA, 519 bp, mouse
  source 1..519: mol_type = other DNA
gaggacctgcgcaacgtcaccccaccaaaggtcagtttgtttgagccatcaaaggcggagatcgccaacaaacagaaagctaccctcgtgtgcttggcccggggcttcttcccagaccacgtagaactttcctggtgggtcaatggaaaggaggttcattccggagtgtgcactgatccccaagcgtacaaggaatccaactatagctactgtctctcatctcggctccgggtgagtgcgacattctggcataatcctcggaaccactttcgatgccaagtgcagtttcatgggttgagcgaggaagacaagtggcccgagggcagtcctaaaccagtcactcaaaacataagcgccgaggcatggggtagagccgattgtgggattactagcgcttcataccaacaaggggtattgagcgctacaattctttacgaaattctcctcggcaaggcgacgctctacgccgtactggtgtctactctcgtggttatggcaatggtgaaacggaaaaacagc

SEQ ID NO: 99 - protein, 9 aa, Artificial Sequence
VVGAGGVGK

SEQ ID NO: 100 - protein, 10 aa, Artificial Sequence
VVVGAGGVGK

SEQ ID NO: 101 - protein, 9 aa, Artificial Sequence
VVGAVGVGK

SEQ ID NO: 102 - protein, 10 aa, Artificial Sequence
VVVGAVGVGK

SEQ ID NO: 103 - protein, 9 aa, Artificial Sequence
VVGADGVGK

SEQ ID NO: 104 - protein, 10 aa, Artificial Sequence
VVVGADGVGK

SEQ ID NO: 105 - protein, 137 aa, mouse
NIQNPEPAVYQLKDPRSQDSTLCLFTDFDSQINVPKTMESGTFITDKCVLDMKAMDSKSNGAIAWSNQTSFTCQDIFKETNATYPSSDVPCDATLTEKSFETDMNLNFQNLSVMGLRILLLKVAGFNLLMTLRLWSS

SEQ ID NO: 106 - protein, 19 aa, Artificial Sequence
MGCRLLCCVVFCLLQAGPL

SEQ ID NO: 107 - protein, 20 aa, Artificial Sequence
MAGIRALFMYLWLQLDWVSR

SEQ ID NO: 108 - protein, 19 aa, Artificial Sequence
MSTRLLCWAALCLLGAELT

SEQ ID NO: 109 - protein, 22 aa, Artificial Sequence
MMKSLRVLLVILWLQLSWVWSQ

SEQ ID NO: 110 - protein, 19 aa, Artificial Sequence
MGPQLLGYVVLCLLGAGPL